European Patent Application EP 4 537 852 A1, published April 16, 2025. Title: HER2-GST-SN-38 복합체 및 이를 포함하는 증식성 질환의 예방 또는 치료용 약학적 조성물. Applicant: 주식회사 케이엠디바이오. Application KR. The sequence listing filed with the application follows.

SEQUENCE LISTING (16 sequences)

SEQ ID NO: 1 - protein, 24 aa, synthetic construct
SGGGSGGGSGGGSGGGSGGGSGGG

SEQ ID NO: 2 - protein, 5 aa, synthetic construct
GGGGS

SEQ ID NO: 3 - protein, 5 aa, synthetic construct
SGGGG

SEQ ID NO: 4 - protein, 5 aa, synthetic construct
SRSSG

SEQ ID NO: 5 - protein, 5 aa, synthetic construct
SGSSC

SEQ ID NO: 6 - protein, 12 aa, synthetic construct
GKSSGSGSESKS

SEQ ID NO: 7 - protein, 6 aa, synthetic construct
RPPPPC

SEQ ID NO: 8 - protein, 7 aa, synthetic construct
SSPPPPC

SEQ ID NO: 9 - protein, 14 aa, synthetic construct
GSTSGSGKSSEGKG

SEQ ID NO: 10 - protein, 18 aa, synthetic construct
GSTSGSGKSSEGSGSTKG

SEQ ID NO: 11 - protein, 18 aa, synthetic construct
GSTSGSGKPGSGEGSTKG

SEQ ID NO: 12 - protein, 14 aa, synthetic construct
EGKSSGSGSESKEF

SEQ ID NO: 13 - protein, 222 aa, synthetic construct
MAEKPKLHYFNARGRMESTRWLLAAAGVEFEEKFIKSAEDLDKLRNDGYLMFQQVPMVEIDGMKLVQTRAILNYIASKYNLYGKDIKERALIDMYIEGIADLGEMILLLPVCPPEEKDAKLALIKEKIKNRYFPAFEKVLKSHGQDYLVGNKLSRADIHLVELLYYVEELDSSLISSFPLLKALKTRISNLPTVKKFLQPGSPRKPPMDEKSLEEARKIFRF

SEQ ID NO: 14 - protein, 58 aa, synthetic construct
VDNKFNKEMRNAYWEIALLPNLNNQQKRAFIRSLYDDPSQSANLLAEAKKLNDAQAPK

SEQ ID NO: 15 - protein, 304 aa, synthetic construct
MAEKPKLHYFNARGRMESTRWLLAAAGVEFEEKFIKSAEDLDKLRNDGYLMFQQVPMVEIDGMKLVQTRAILNYIASKYNLYGKDIKERALIDMYIEGIADLGEMILLLPVCPPEEKDAKLALIKEKIKNRYFPAFEKVLKSHGQDYLVGNKLSRADIHLVELLYYVEELDSSLISSFPLLKALKTRISNLPTVKKFLQPGSPRKPPMDEKSLEEARKIFRFSGGGSGGGSGGGSGGGSGGGSGGGVDNKFNKEMRNAYWEIALLPNLNNQQKRAFIRSLYDDPSQSANLLAEAKKLNDAQAPK

SEQ ID NO: 16 - DNA, 915 bp, synthetic construct
  source 1..915: mol_type = other DNA
atggcagaaaaaccgaaactgcattatttcaatgcacgtggtcgtatggaaagcacccgttggctgctggcagccgcaggcgttgaatttgaagaaaaattcattaaaagcgcagaagatctggacaaactgcgcaatgatggttatctgatgtttcagcaggttccgatggttgaaattgatggtatgaaactggttcagacccgtgcaattctgaactatattgccagcaaatataacctgtacggcaaggatattaaagaacgtgcactgatcgatatgtacattgaaggtattgcagatctgggcgaaatgattctgctgctgccggtttgtcctccggaagaaaaagatgcaaaactggcactgatcaaagagaaaatcaagaaccgttattttccggcatttgaaaaggttctgaaaagtcatggtcaggattatctggtgggtaataaactgagccgtgcagatattcatctggttgaactgctgtattatgtggaagaactggatagcagcctgattagcagctttccgctgctgaaagcactgaaaacccgtattagcaatctgccgaccgtgaaaaaattcctgcagcctggtagtccgcgtaaaccgcctatggatgaaaaaagcctggaagaagcacgtaaaatctttcgttttagcggtggtggttcaggtggtggtagcggtggcggtagtggcggtggcagtggcggaggttctggtggcggtgttgataacaaatttaacaaagaaatgcgcaacgcctattgggaaattgcactgctgccgaatctgaataatcagcagaaacgtgcatttatccgtagcctgtatgatgatccgagccagagcgcaaatctgctggccgaagcaaaaaaactgaatgatgcacaggcaccgaaataa